European Patent Application EP 4 692 293 A1, published February 11, 2026. Title: Composition. Applicant: Unilever IP Holdings B.V. The sequence listing filed with the application follows.

SEQUENCE LISTING (4 sequences)

SEQ ID NO: 1 - protein, 257 aa, Pyrococcus furiosus
MTQVYKAKFGTPNRGWVIIVHGLGEHSGRYSKLVSMLVNEGYAVYTFDWPGHGKSPGKRGHTSVEEAMEIIDFIIEEINDKPFLFGHSLGGLTVIRYAETRPEKIRGVIASSPALAKSPKTPSFMVALAKILGVLLPSLTLSNGIDPNLLSRNPDAVKRYIEDPLVHDRISAKLGRSIFKNMDLAHREAHKIKVPVLLLVGTGDVITPPEGARKLYGEIKVEDKEIVEFEGAYHEIFEDPFWGEEFHKKIVEWIKKH

SEQ ID NO: 2 - protein, 263 aa, Pyrococcus furiosus
MTQVYKAKFGTPNRGWVIIVHGLGEHSGRYSKLVSMLVNEGYAVYTFDWPGHGKSPGKRGHTSVEEAMEIIDFIIEEINDKPWRKRFLFGHSLGGLTVIRYAETRPEKIRGVIASSPALAKSPKTPSFMVALAKILGVLLPSLTLSNGIDPNLLSRNPDAVKRYIEDPLVHDRISAKLGRSIFKNMDLAHREAHKIKVPVLLLVGTGDVITPPEGARKLYGEIKVEDKEIVEFEGAYHEIFEDPFWGEEFHKKIVEWIKKHLE

SEQ ID NO: 3 - protein, 266 aa, Pyrococcus furiosus
MTQVYKAKFGTPNRGWVIIVHGLGEHSGRYSKLVSMLVNEGYAVYTFDWPGHGKSPGKRGHTSVEEAMEIIDFIIELAAFWQQEINDKPFLFGHSLGGLTVIRYAETRPEKIRGVIASSPALAKSPKTPSFMVALAKILGVLLPSLTLSNGIDPNLLSRNPDAVKRYIEDPLVHDRISAKLGRSIFKNMDLAHREAHKIKVPVLLLVGTGDVITPPEGARKLYGEIKVEDKEIVEFEGAYHEIFEDPFWGEEFHKKIVEWIKKHLE

SEQ ID NO: 4 - protein, 270 aa, Pyrococcus furiosus
MTQVYKAKFGTPNRGWVIIVHGLGEHSGRYSKLVSMLVNEGYAVYTFDWPGHGKSPGKRGDLGFFGEEHPVHTSVEEAMEIIDFIIEEINDKPFLFGHSLGGLTVIRYAETRPEKIRGVIASSPALAKSPKTPSFMVALAKILGVLLPSLTLSNGIDPNLLSRNPDAVKRYIEDPLVHDRISAKLGRSIFKNMDLAHREAHKIKVPVLLLVGTGDVITPPEGARKLYGEIKVEDKEIVEFEGAYHEIFEDPFWGEEFHKKIVEWIKKHLE